European Patent Application EP 4 541 191 A1, published April 23, 2025. Title: MARINE STREPTOMYCES AS NATURAL ANTIFUNGAL AGENTS TO COMBAT THE CHESTNUT BROWN ROT FUNGUS GNOMONIOPSIS SMITHOGILVYI. Applicant: CIIMAR – CENTRO INTERDISCIPLINAR DE INVESTIGAÇÃO MARINHA E AMBIENTAL. The sequence listing filed with the application follows.

SEQUENCE LISTING (13 sequences)

SEQ ID NO: 1 - RNA, 1399 nt, Streptomyces sp.
  source 1..1399: mol_type = other RNA
ccatgcagtcggacgatgaccgctttcgggcggggattagtggcgaacgggtgagtaacacgtgggcaatctgccctgcactctgggacaagccctggaaacggggtctaataccggatatgactgtccatcgcatggtggatggtgtaaagctccggcggtgcaggatgagcccgcggcctatcagcttgttggtgaggtagtggctcaccaaggcgacgacgggtagccggcctgagagggcgaccggccacactgggactgagacacggcccagactcctacgggaggcagcagtggggaatattgcacaatgggcgaaagcctgatgcagcgacgccgcgtgagggatgacggccttcgggttgtaaacctctttcagcagggaagaagcgaaagtgacggtacctgcagaagaagcgccggctaactacgtgccagcagccgcggtaatacgtagggcgcaagcgttgtccggaattattgggcgtaaagagctcgtaggcggcttgtcacgtcggttgtgaaagcccggggcttaaccccgggtctgcagtcgatacgggcaggctagagttcggtaggggagatcggaattcctggtgtagcggtgaaatgcgcagatatcaggaggaacaccggtggcgaaggcggatctctgggccgatactgacgctgaggagcgaaagcgtggggagcgaacaggattagataccctggtagtccacgccgtaaacggtgggcactaggtgtgggcaacattccacgttgtccgtgccgcagctaacgcattaagtgccccgcctggggagtacggccgcaaggctaaaactcaaaggaattgacgggggcccgcacaagcggcggagcatgtggcttaattcgacgcaacgcgaagaaccttaccaaggcttgacatacaccggaaacgtctggagacaggcgcccccttgtggtcggtgtacaggtggtgcatggctgtcgtcagctcgtgtcgtgagatgttgggttaagtcccgcaacgagcgcaacccttgtcccgtgttgccagcaggcccttgtggtgctggggactcacgggagaccgccggggtcaactcggaggaaggtggggacgacgtcaagtcatcatgccccttatgtcttgggctgcacacgtgctacaatggccggtacaatgagctgcgataccgcgaggtggagcgaatctcaaaaagccggtctcagttcggattggggtctgcaactcgaccccatgaagtcggagtcgctagtaatcgcagatcagcattgctgcggtgaatacgttcccgggccttgtacacaccgcccgtcacgtcacgaaagtcggtaacacccgaagccggtggcccaacccctgtgggagggagctgttcga

SEQ ID NO: 2 - RNA, 1376 nt, Streptomyces sp.
  source 1..1376: mol_type = other RNA
catgcagtcgacgatgaccgctttcgggcggggattagtggcgaacgggtgagtaacacgtgggcaatctgccctgcactctgggacaagccctggaaacggggtctaataccggatatgactgtccatcgcatggtggatggtgtaaagctccggcggtgcaggatgagcccgcggcctatcagcttgttggtgaggtagtggctcaccaaggcgacgacgggtagccggcctgagagggcgaccggccacactgggactgagacacggcccagactcctacgggaggcagcagtggggaatattgcacaatgggcgaaagcctgatgcagcgacgccgcgtgagggatgacggccttcgggttgtaaacctctttcagcagggaagaagcgaaagtgacggtacctgcagaagaagcgccggctaactacgtgccagcagccgcggtaatacgtagggcgcaagcgttgtccggaattattgggcgtaaagagctcgtaggcggcttgtcacgtcggttgtgaaagcccggggcttaaccccgggtctgcagtcgatacgggcaggctagagttcggtaggggagatcggaattcctggtgtagcggtgaaatgcgcagatatcaggaggaacaccggtggcgaaggcggatctctgggccgatactgacgctgaggagcgaaagcgtggggagcgaacaggattagataccctggtagtccacgccgtaaacggtgggcactaggtgtgggcaacattccacgttgtccgtgccgcagctaacgcattaagtgccccgcctggggagtacggccgcaaggctaaaactcaaaggaattgacgggggcccgcacaagcggcggagcatgtggcttaattcgacgcaacgcgaagaaccttaccaaggcttgacatacaccggaaacgtctggagacaggcgcccccttgtggtcggtgtacaggtggtgcatggctgtcgtcagctcgtgtcgtgagatgttgggttaagtcccgcaacgagcgcaacccttgtcccgtgttgccagcaggcccttgtggtgctggggactcacgggagaccgccggggtcaactcggaggaaggtggggacgacgtcaagtcatcatgccccttatgtcttgggctgcacacgtgctacaatggccggtacaatgagctgcgataccgcgaggtggagcgaatctcaaaaagccggtctcagttcggattggggtctgcaactcgaccccatgaagtcggagtcgctagtaatcgcagatcagcattgctgcggtgaatacgttcccgggccttgtacacaccgcccgtcacgtcacgaaagtcggtaacacccgaagccggggcccaacccc

SEQ ID NO: 3 - RNA, 1364 nt, Streptomyces sp.
  source 1..1364: mol_type = other RNA
gctttcgggcggggattagtggcgaacgggtgagtaacacgtgggcaatctgccctgcactctgggacaagccctggaaacggggtctaataccggatatgactgtccatcgcatggtggatggtgtaaagctccggcggtgcaggatgagcccgcggcctatcagcttgttggtgaggtagtggctcaccaaggcgacgacgggtagccggcctgagagggcgaccggccacactgggactgagacacggcccagactcctacgggaggcagcagtggggaatattgcacaatgggcgaaagcctgatgcagcgacgccgcgtgagggatgacggccttcgggttgtaaacctctttcagcagggaagaagcgaaagtgacggtacctgcagaagaagcgccggctaactacgtgccagcagccgcggtaatacgtagggcgcaagcgttgtccggaattattgggcgtaaagagctcgtaggcggcttgtcacgtcggttgtgaaagcccggggcttaaccccgggtctgcagtcgatacgggcaggctagagttcggtaggggagatcggaattcctggtgtagcggtgaaatgcgcagatatcaggaggaacaccggtggcgaaggcggatctctgggccgatactgacgctgaggagcgaaagcgtggggagcgaacaggattagataccctggtagtccacgccgtaaacggtgggcactaggtgtgggcaacattccacgttgtccgtgccgcagctaacgcattaagtgccccgcctggggagtacggccgcaaggctaaaactcaaaggaattgacgggggcccgcacaagcggcggagcatgtggcttaattcgacgcaacgcgaagaaccttaccaaggcttgacatacaccggaaacgtctggagacaggcgcccccttgtggtcggtgtacaggtggtgcatggctgtcgtcagctcgtgtcgtgagatgttgggttaagtcccgcaacgagcgcaacccttgtcccgtgttgccagcaggcccttgtggtgctggggactcacgggagaccgccggggtcaactcggaggaaggtggggacgacgtcaagtcatcatgccccttatgtcttgggctgcacacgtgctacaatggccggtacaatgagctgcgataccgcgaggtggagcgaatctcaaaaagccggtctcagttcggattggggtctgcaactcgaccccatgaagtcggagtcgctagtaatcgcagatcagcattgctgcggtgaatacgttcccgggccttgtacacaccgcccgtcacgtcacgaaagtcggtaacacccgaagccggtggcccaaccccttgtgg

SEQ ID NO: 4 - RNA, 1346 nt, Streptomyces sp.
  source 1..1346: mol_type = other RNA
ccgctttcgggcggggattagtggcgaacgggtgagtaacacgtgggcaatctgccctgcactctgggacaagccctggaaacggggtctaataccggatatgactgtccatcgcatggtggatggtgtaaagctccggcggtgcaggatgagcccgcggcctatcagcttgttggtgaggtagtggctcaccaaggcgacgacgggtagccggcctgagagggcgaccggccacactgggactgagacacggcccagactcctacgggaggcagcagtggggaatattgcacaatgggcgaaagcctgatgcagcgacgccgcgtgagggatgacggccttcgggttgtaaacctctttcagcagggaagaagcgaaagtgacggtacctgcagaagaagcgccggctaactacgtgccagcagccgcggtaatacgtagggcgcaagcgttgtccggaattattgggcgtaaagagctcgtaggcggcttgtcacgtcggttgtgaaagcccggggcttaaccccgggtctgcagtcgatacgggcaggctagagttcggtaggggagatcggaattcctggtgtagcggtgaaatgcgcagatatcaggaggaacaccggtggcgaaggcggatctctgggccgatactgacgctgaggagcgaaagcgtggggagcgaacaggattagataccctggtagtccacgccgtaaacggtgggcactaggtgtgggcaacattccacgttgtccgtgccgcagctaacgcattaagtgccccgcctggggagtacggccgcaaggctaaaactcaaaggaattgacgggggcccgcacaagcggcggagcatgtggcttaattcgacgcaacgcgaagaaccttaccaaggcttgacatacaccggaaacgtctggagacaggcgcccccttgtggtcggtgtacaggtggtgcatggctgtcgtcagctcgtgtcgtgagatgttgggttaagtcccgcaacgagcgcaacccttgtcccgtgttgccagcaggcccttgtggtgctggggactcacgggagaccgccggggtcaactcggaggaaggtggggacgacgtcaagtcatcatgccccttatgtcttgggctgcacacgtgctacaatggccggtacaatgagctgcgataccgcgaggtggagcgaatctcaaaaagccggtctcagttcggattggggtctgcaactcgaccccatgaagtcggagtcgctagtaatcgcagatcagcattgctgcggtgaatacgttcccgggccttgtacacaccgcccgtcacgtcacgaaagtcggtaacacccgaagcc

SEQ ID NO: 5 - RNA, 1391 nt, Streptomyces resistomycificus
  source 1..1391: mol_type = other RNA
tgcagtcgaacgatgaaccgctttcgggcggggattagtggcgaacgggtgagtaacacgtgggcaatctgccctgcactctgggacaagccctggaaacggggtctaataccggatatgactgtccatcgcatggtggatggtgtaaagctccggcggtgcaggatgagcccgcggcctatcagcttgttggtgaggtagtggctcaccaaggcgacgacgggtagccggcctgagagggcgaccggccacactgggactgagacacggcccagactcctacgggaggcagcagtggggaatattgcacaatgggcgaaagcctgatgcagcgacgccgcgtgagggatgacggccttcgggttgtaaacctctttcagcagggaagaagcgaaagtgacggtacctgcagaagaagcgccggctaactacgtgccagcagccgcggtaatacgtagggcgcaagcgttgtccggaattattgggcgtaaagagctcgtaggcggcttgtcacgtcggttgtgaaagcccggggcttaaccccgggtctgcagtcgatacgggcaggctagagttcggtaggggagatcggaattcctggtgtagcggtgaaatgcgcagatatcaggaggaacaccggtggcgaaggcggatctctgggccgatactgacgctgaggagcgaaagcgtggggagcgaacaggattagataccctggtagtccacgccgtaaacggtgggcactaggtgtgggcaacattccacgttgtccgtgccgcagctaacgcattaagtgccccgcctggggagtacggccgcaaggctaaaactcaaaggaattgacgggggcccgcacaagcggcggagcatgtggcttaattcgacgcaacgcgaagaaccttaccaaggcttgacatacaccggaaacgtctggagacaggcgcccccttgtggtcggtgtacaggtggtgcatggctgtcgtcagctcgtgtcgtgagatgttgggttaagtcccgcaacgagcgcaacccttgtcccgtgttgccagcaggcccttgtggtgctggggactcacgggagaccgccggggtcaactcggaggaaggtggggacgacgtcaagtcatcatgccccttatgtcttgggctgcacacgtgctacaatggccggtacaatgagctgcgataccgcgaggtggagcgaatctcaaaaagccggtctcagttcggattggggtctgcaactcgaccccatgaagtcggagtcgctagtaatcgcagatcagcattgctgcggtgaatacgttcccgggccttgtacacaccgcccgtcacgtcacgaaagtcggtaacacccgaagccggtggcccaaccccttgtgggagggagc

SEQ ID NO: 6 - RNA, 1391 nt, Streptomyces sp.
  source 1..1391: mol_type = other RNA
catgcagtcgaacgatgaagcccttcggggtggattagtggcgaacgggtgagtaacacgtgggcaatctgccctgcactctgggacaagccctggaaacggggtctaataccggatatgactgtccaccgcatggtggatggtgtaaagctccggcggtgcaggatgagcccgcggcctatcanctngttggtgaggtagtggctcaccaaggcgacgacgggtagccggcctgagagggcgaccggccacactgggactgagacacggcccagactcctacgggaggcagcagtggggaatattgcacaatgggcgaaagcctgatgcagcgacgccgcgtgagggatgacggccttcgggttgtaaacctctttcagcagggaagaagcgaaagtgacggtacctgcagaagaagcgccggctaactacgtgccagcagccgcggtaatacgtagggcgcaagcgttgtccggaattattgggcgtaaagagctcgtaggcggcttgtcacgtcggttgtgaaagcccggggcttaaccccgggtctgcagtcgatacgggcaggctagagttcggtaggggagatcggaattcctggtgtagcggtgaaatgcgcagatatcaggaggaacaccggtggcgaaggcggatctctgggccgatactgacgctgaggagcgaaagcgtggggagcgaacaggattagataccctggtagtccacgccgtaaacggtgggcactaggtgtgggcaacattccacgttgtccgtgccgcagctaacgcattaagtgccccgcctggggagtacggccgcaaggctaaaactcaaaggaattgacgggggcccgcacaagcggcggagcatgtggcttaattcgacgcaacgcgaagaaccttaccaaggcttgacatacaccggaaagcatcagagatggtgccccccttgtggtcggtgtacaggtggtgcatggctgtcgtcagctcgtgtcgtgagatgttgggttaagtcccgcaacgagcgcaacccttgtcccgtgttgccagcaggcccttgtggtgctggggactcacgggagaccgccggggtcaactcggaggaaggtggggacgacgtcaagtcatcatgccccttatgtcttgggctgcacacgtgctacaatggccggtacaatgagctgcgataccgcgaggtggagcgaatctcaaaaagccggtctcagttcggattggggtctgcaactcgaccccatgaagtcggagtcgctagtaatcgcagatcagcattgctgcggtgaatacgttcccgggccttgtacacaccgcccgtcacgtcacgaaagtcggtaacacccgaagccggtggcccaaccccttgtgggagggagc

SEQ ID NO: 7 - RNA, 1388 nt, Streptomyces sp.
  source 1..1388: mol_type = other RNA
agtcgaacgatgaaccgctttcgggcggggattagtggcgaacgggtgaataacacgtgggcaatctgccctgcactctgggacaagccctggaaacggggtctaataccggatatgactgtccatcgcatggtggatggtgtaaagctccggcggtgcaggatgagcccgcggcctatcagcttgttggtgaggtagtggctcaccaaggcgacgacgggtagccggcctgagagggcgaccggccacactgggactgagacacggcccagactcctacgggaggcagcagtggggaatattgcacaatgggcgaaagcctgatgcagcgacgccgcgtgagggatgacggccttcgggttgtaaacctctttcagcagggaagaagcgaaagtgacggtacctgcagaagaagcgccggctaactacgtgccagcagccgcggtaatacgtagggcgcaagcgttgtccggaattattgggcgtaaagagctcgtaggcggcttgtcacgtcggttgtgaaagcccggggcttaaccccgggtctgcagtcgatacgggcaggctagagttcggtaggggagatcggaattcctggtgtagcggtgaaatgcgcagatatcaggaggaacaccggtggcgaaggcggatctctgggccgatactgacgctgaggagcgaaagcgtggggagcgaacaggattagataccctggtagtccacgccgtaaacggtgggcactaggtgtgggcaacattccacgttgtccgtgccgcagctaacgcattaagtgccccgcctggggagtacggccgcaaggctaaaactcaaaggaattgacgggggcccgcacaagcggcggagcatgtggcttaattcgacgcaacgcgaagaaccttaccaaggcttgacatacaccggaaacgtctggagacaggcgcccccttgtggtcggtgtacaggtggtgcatggctgtcgtcagctcgtgtcgtgagatgttgggttaagtcccgcaacgagcgcaacccttgtcccgtgttgccagcaggcccttgtggtgctggggactcacgggagaccgccggggtcaactcggaggaaggtggggacgacgtcaagtcatcatgccccttatgtcttgggctgcacacgtgctacaatggccggtacaatgagctgcgataccgcgaggtggagcgaatctcaaaaagccggtctcagttcggattggggtctgcaactcgaccccatgaagtcggagtcgctagtaatcgcagatcagcattgctgcggtgaatacgttcccgggccttgtacacaccgcccgtcacgtcacgaaagtcggtaacacccgaagccggtggcccaaccccttgtgggagggagc

SEQ ID NO: 8 - RNA, 1378 nt, Strptomyces sp.
  source 1..1378: mol_type = other RNA
atgaaccgctttcgggcggggattagtggcgaacgggtgagtaacacgtgggcaatctgccctgcactctgggacaagccctggaaacggggtctaataccggatatgactgtccatcgcatggtggatggtgtaaagctccggcggtgcaggatgagcccgcggcctatcagcttgttggtgaggtagtggctcaccaaggcgacgacgggtagccggcctgagagggcgaccggccacactgggactgagacacggcccagactcctacgggaggcagcagtggggaatattgcacaatgggcgaaagcctgatgcagcgacgccgcgtgagggatgacggccttcgggttgtaaacctctttcagcagggaagaagcgaaagtgacggtacctgcagaagaagcgccggctaactacgtgccagcagccgcggtaatacgtagggcgcaagcgttgtccggaattattgggcgtaaagagctcgtaggcggcttgtcacgtcggttgtgaaagcccggggcttaaccccgggtctgcagtcgatacgggcaggctagagttcggtaggggagatcggaattcctggtgtagcggtgaaatgcgcagatatcaggaggaacaccggtggcgaaggcggatctctgggccgatactgacgctgaggagcgaaagcgtggggagcgaacaggattagataccctggtagtccacgccgtaaacggtgggcactaggtgtgggcaacattccacgttgtccgtgccgcagctaacgcattaagtgccccgcctggggagtacggccgcaaggctaaaactcaaaggaattgacgggggcccgcacaagcggcggagcatgtggcttaattcgacgcaacgcgaagaaccttaccaaggcttgacatacaccggaaacgtctggagacaggcgcccccttgtggtcggtgtacaggtggtgcatggctgtcgtcagctcgtgtcgtgagatgttgggttaagtcccgcaacgagcgcaacccttgtcccgtgttgccagcaggcccttgtggtgctggggactcacgggagaccgccggggtcaactcggaggaaggtggggacgacgtcaagtcatcatgccccttatgtcttgggctgcacacgtgctacaatggccggtacaatgagctgcgataccgcgaggtggagcgaatctcaaaaagccggtctcagttcggattggggtctgcaactcgaccccatgaagtcggagtcgctagtaatcgcagatcagcattgctgcggtgaatacgttcccgggccttgtacacaccgcccgtcacgtcacgaaagtcggtaacacccgaagccggtggcccaaccccttgtgggagggag

SEQ ID NO: 9 - RNA, 1379 nt, Streptomyces sp.
  source 1..1379: mol_type = other RNA
atgaaccgctttcgggcggggattagtggcgaacgggtgagtaacacgtgggcaatctgccctgcactctgggacaagccctggaaacggggtctaataccggatatgaccgtctgccgcatggtggatggtgtaaagctccggcggtgcaggatgagcccgcggcctatcagcttgttggtgaggtagtggctcaccaaggcgacgacgggtagccggcctgagagggcgaccggccacactgggactgagacacggcccagactcctacgggaggcagcagtggggaatattgcacaatgggcgaaagcctgatgcagcgacgccgcgtgagggatgacggccttcgggttgtaaacctctttcagcagggaagaagcgaaagtgacggtacctgcagaagaagcgccggctaactacgtgccagcagccgcggtaatacgtagggcgcaagcgttgtccggaattattgggcgtaaagagctcgtaggcggcttgtcacgtcggttgtgaaagcccggggcttaaccccgggtctgcagtcgatacgggcaggctagagttcggtaggggagatcggaattcctggtgtagcggtgaaatgcgcagatatcaggaggaacaccggtggcgaaggcggatctctgggccgatactgacgctgaggagcgaaagcgtggggagcgaacaggattagataccctggtagtccacgccgtaaacggtgggcactaggtgtgggcaacattccacgttgtccgtgccgcagctaacgcattaagtgccccgcctggggagtacggccgcaaggctaaaactcaaaggaatttgacgggggcccgcacaagcggcggagcatgtggcttaattcgacgcaacgcgaagaaccttaccaaggcttgacatacaccggaaacgtctggagacaggcgcccccttgtggtcggtgtacaggtggtgcatggctgtcgtcagctcgtgtcgtgagatgttgggttaagtcccgcaacgagcgcaacccttgtcccgtgttgccagcaggcccttgtggtgctggggactcacgggagaccgccggggtcaactcggaggaaggtggggacgacgtcaagtcatcatgccccttatgtcttgggctgcacacgtgctacaatggccggtacaatgagctgcgataccgtgaggtggagcgaatctcaaaaagccggtctcagttcggattggggtctgcaactcgaccccatgaagtcggagtcgctagtaatcgcagatcagcattgctgcggtgaatacgttcccgggccttgtacacaccgcccgtcacgtcacgaaagtcggtaacacccgaagccggtggcccaaccccttgtgggagggag

SEQ ID NO: 10 - RNA, 1362 nt, Streptomyces sp.
  source 1..1362: mol_type = other RNA
atcagtggcgaacgggtgagtaacacgtgagcaatctgcccctgactctgggacaagcgcctggaaacggcgtctaataccggatatgaactggatcccgcatggttacggggtggaaagatctgtcggtgaaggatgagctcgcggcctatcagcttgttggtgaggtaatggctcaccaaggcgtcgacgggtagccggcctgagagggtgaccggccacactgggactgagacacggcccagactcctacgggaggcagcagtggggaatattgcacaatgggcgaaagcctgatgcagcgacgccgcgtgagggatgacggccttcgggttgtaaacctctttcagcagggaagaagcgaaagtgacggtacctgcagaagaagcgccggctaactacgtgccagcagccgcggtaatacgtagggcgcaagcgttgtccggaattattgggcgtaaagagctcgtaggcggcttgtcacgtcggatgtgaaagcccggggcttaaccccgggtctgcattcgatacgggctagctagagtgtggtaggggagatcggaattcctggtgtagcggtgaaatgcgcagatatcaggaggaacaccggtggcgaaggcggatctctgggccattactgacgctgaggagcgaaagcgtggggagcgaacaggattagataccctggtagtccacgccgtaaacgttgggaactaggtgttggcgacattccacgtngtcggtgccgcagctaacgcattaagttccccgcctggggagtacggccgcaaggctaaaactcaaaggaattgacgggggcccgcacaagcagcggagcatgtggcttaattcgacgcaacgcgaagaaccttaccaaggcttgacatataccggaaagcatcagagatggtgccccccttgtggtcggtatacaggtggtgcatggctgtcgtcagctcgtgtcgtgagatgttgggttaagtcccgcaacgagcgcaacccttgttctgtgttgccagcatgcccttcggggtgatggggactcacaggagactgccggggtcaactcggaggaaggtggggacgacgtcaagtcatcatgccccttatgtcttgggctgcacacgtgctacaatggccggtacaatgagctgcgatgccgcgaggcggagcgaatctcaaaaagccggtctcagttcggattggggtctgcaactcgaccccatgaagtcggagttgctagtaatcgcagatcagcattgctgcggtgaatacgttcccgggccttgtacacaccgcccgtcacgtcacgaaagtcggtaacacccgaagccggtggcccaaccccttgtgggagggagc

SEQ ID NO: 11 - RNA, 1381 nt, Streptomyces sp.
  source 1..1381: mol_type = other RNA
cgatgaaccgctttcgggcggggattagtggcgaacgggtgagtaacacgtgggcaatctgccctgcactctgggacaagccctggaaacggggtctaataccggatatgactgtccatcgcatggtggatggtgtaaagctccggcggtgcaggatgagcccgcggcctatcagcttgttggtgaggtagtggctcaccaaggcgacgacgggtagccggcctgagagggcgaccggccacactgggactgagacacggcccagactcctacgggaggcagcagtggggaatattgcacaatgggcgaaagcctgatgcagcgacgccgcgtgagggatgacggccttcgggttgtaaacctctttcagcagggaagaagcgaaagtgacggtacctgcagaagaagcgccggctaactacgtgccagcagccgcggtaatacgtagggcgcaagcgttgtccggaattattgggcgtaaagagctcgtaggcggcttgtcacgtcggttgtgaaagcccggggcttaaccccgggtctgcagtcgatacgggcaggctagagttcggtaggggagatcggaattcctggtgtagcggtgaaatgcgcagatatcaggaggaacaccggtggcgaaggcggatctctgggccgatactgacgctgaggagcgaaagcgtggggagcgaacaggattagataccctggtagtccacgccgtaaacggtgggcactaggtgtgggcaacattccacgttgtccgtgccgcagctaacgcattaagtgccccgcctggggagtacggccgcaaggctaaaactcaaaggaattgacgggggcccgcacaagcggcggagcatgtggcttaattcgacgcaacgcgaagaaccttaccaaggcttgacatacaccggaaacgtctggagacaggcgcccccttgtggtcggtgtacaggtggtgcatggctgtcgtcagctcgtgtcgtgagatgttgggttaagtcccgcaacgagcgcaacccttgtcccgtgttgccagcaggcccttgtggtgctggggactcacgggagaccgccggggtcaactcggaggaaggtggggacgacgtcaagtcatcatgccccttatgtcttgggctgcacacgtgctacaatggccggtacaatgagctgcgataccgngaggtggagcgaatctcaaaaagccggtctcagttcggattggggtctgcaactcgaccccatgaagtcggagtcgctagtaatcgcagatcagcattgctgcggtgaatacgttcccgggccttgtacacaccgcccgtcacgtcacgaaagtcggtaacacccgaagccggtggcccaaccccttgtgggagggagc

SEQ ID NO: 12 - RNA, 1391 nt, Strptomyces sp.
  source 1..1391: mol_type = other RNA
tgcagtcgaacgatgaagcccttcggggtggattagtggcgaacgggtgagtaacacgtgggcaatctgccctgcactctgggacaagccctggaaacggggtctaataccggatatgaccgtccatcgcatggtggatggtgtaaagctccggcggtgcaggatgagcccgcggcctatcagctagttggtgaggtagtggctcaccaaggcgacgacgggtagccggcctgagagggcgaccggccacactgggactgagacacggcccagactcctacgggaggcagcagtggggaatattgcacaatgggcgaaagcctgatgcagcgacgccgcgtgagggatgacggccttcgggttgtaaacctctttcagcagggaagaagcgaaagtgacggtacctgcagaagaagcgccggctaactacgtgccagcagccgcggtaatacgtagggcgcaagcgttgtcccggaattattgggcgtaaagagctcgtaggcggcttgtcacgtcggttgtgaaagcccggggcttaaccccgggtctgcagtcgatacgggcaggctagagtttcggtaggggagatcggaattcctggtgtagcggtgaaatgcgcagatatcaggaggaacaccggtggcgaaggcggatctctgggccgatactgacgctgaggagcgaaagcgtggggagcgaacaggattagataccctggtagtccacgccgtaaacggtgggcactaggtgtgggcaacattccacgttgtccgtgccgcagctaacgcattaagtgccccgcctggggagtacggccgcaaggctaaaactcaaaggaattgacgggggcccgcacaagcggcggagcatgtggcttaattcgacgcaacgcgaagaaccttaccaaggcttgacatacaccggaaagcatcagagatggtgccccccttgtggtcggtgtacaggtggtgcatggctgtcgtcagctcgtgtcgtgagatgttgggttaagtcccgcaacgagcgcaacccttgtcccgtgttgccagcaggcccttgtggtgctggggactcacgggagaccgccggggtcaactcggaggaaggtggggacgacgtcaagtcatcatgccccttatgtcttgggctgcacacgtgctacaatggccggtacaatgagctgcgataccgtgaggtggagcgaatctcaaaaagccggtctcagttcggattggggtctgcaactcgaccccatgaagtcggagtcgctagtaatcgcagatcagcattgctgcggtgaatacgttcccgggccttgtacacaccgcccgtcacgtcacgaaagtcggtaacacccgaagccggtggcccaacccccttgtggggaggga

SEQ ID NO: 13 - RNA, 1388 nt, Streptomyces sp.
  source 1..1388: mol_type = other RNA
gcagtcgaacgatgaaccgctttcgggcggggattagtggcgaacgggtgagtaacacgtgggcaatctgccctgcactctgggacaagccctggaaacggggtctaataccggatatgactgtccatcgcatggtggatggtgtaaagctccggcggtgcaggatgagcccgcggcctatcagcttgttggtgaggtagtggctcaccaaggcgacgacgggtagccggcctgagagggcgaccggccacactgggactgagacacggcccagactcctacgggaggcagcagtggggaatattgcacaatgggcgaaagcctgatgcagcgacgccgcgtgagggatgacggccttcgggttgtaaacctctttcagcagggaagaagcgaaagtgacggtacctgcagaagaagcgccggctaactacgtgccagcagccgcggtaatacgtagggcgcaagcgttgtccggaattattgggcgtaaagagctcgtaggcggcttgtcacgtcggttgtgaaagcccggggcttaaccccgggtctgcagtcgatacgggcaggctagagttcggtaggggagatcggaattcctggtgtagcggtgaaatgcgcagatatcaggaggaacaccggtggcgaaggcggatctctgggccgatactgacgctgaggagcgaaagcgtggggagcgaacaggattagataccctggtagtccacgccgtaaacggtgggcactaggtgtgggcaacattccacgttgtccgtgccgcagctaacgcattaagtgccccgcctggggagtacggccgcaaggctaaaactcaaaggaattgacgggggcccgcacaagcggcggagcatgtggcttaattcgacgcaacgcgaagaaccttaccaaggcttgacatacaccggaaacgtctggagacaggcgcccccttgtggtcggtgtacaggtggtgcatggctgtcgtcagctcgtgtcgtgagatgttgggttaagtcccgcaacgagcgcaacccttgtcccgtgttgccagcaggcccttgtggtgctggggactcacgggagaccgccggggtcaactcggaggaaggtggggacgacgtcaagtcatcatgccccttatgtcttgggctgcacacgtgctacaatggccggtacaatgagctgcgataccgcgaggtggagcgaatctcaaaaagccggtctcagttcggattggggtctgcaactcgaccccatgaagtcggagtcgctagtaatcgcagatcagcattgctgcggtgaatacgttcccgggccttgtacacaccgcccgtcacgtcacgaaagtcggtaacacccgaagccggtggcccaaccccttgtgggaggga